European Patent Application EP 4 759 365 A1, published June 17, 2026. Title: NEW FUSION PROTEIN AGAINST ANGIOGENESIS. Applicant: 三鈺生物科技股份有限公司. Application US. The sequence listing filed with the application follows.

SEQUENCE LISTING (8 sequences)

SEQ ID NO: 1 - protein, 126 aa, Homo sapiens
EVQLVESGGGLVQPGRSLRLSCAASGFTFDDYAMHWVRQAPGKGLEWVSGISWNSGSIGYADSVKGRFTISRDNAKNSLYLQMNSLRAEDTALYYCAKDIGGIVGAATLGDAFDIWGQGTMVTVSS

SEQ ID NO: 2 - protein, 106 aa, Homo sapiens
SYELTQPPSVSVSPGQTASITCSGDELGEKYASWYQQKPGQSPVLVIYQDSKRPSGIPERFSGSNSGNTATLTISGTQAMDEADYYCQAWDSSTAVFGGGTKLTVL

SEQ ID NO: 3 - protein, 234 aa, Homo sapiens
EVQLVESGGGLVQPGRSLRLSCAASGFTFDDYAMHWVRQAPGKGLEWVSGISWNSGSIGYADSVKGRFTISRDNAKNSLYLQMNSLRAEDTALYYCAKDIGGIVGAATLGDAFDIWGQGTMVTVSSASTKGPSVFPLAPSSKSTSGGTAALGCLVKDYFPEPVTVSWNSGALTSGVHTFPAVLQSSGLYSLSSVVTVPSSSLGTQTYICNVNHKPSNTKVDKKVEPKSCDKTHT

SEQ ID NO: 4 - protein, 212 aa, Homo sapiens
SYELTQPPSVSVSPGQTASITCSGDELGEKYASWYQQKPGQSPVLVIYQDSKRPSGIPERFSGSNSGNTATLTISGTQAMDEADYYCQAWDSSTAVFGGGTKLTVLGQPKAAPSVTLFPPSSEELQANKATLVCLISDFYPGAVTVAWKADSSPVKAGVETTTPSKQSNNKYAASSYLSLTPEQWKSHRSYSCQVTHEGSTVEKTVAPAECS

SEQ ID NO: 5 - protein, 16 aa, Homo sapiens
GGGGGSGGGGSGGGGS

SEQ ID NO: 6 - protein, 245 aa, Homo sapiens
EVQLVESGGGLVQPGGSLRLSCAASGYDFTHYGMNWVRQAPGKCLEWVGWINTYTGEPTYAADFKRRFTFSLDTSKSTAYLQMNSLRAEDTAVYYCAKYPYYYGTSHWYFDVWGQGTLVTVSSGGGGSGGGGSGGGGSDIQLTQSPSSLSASVGDRVTITCSASQDISNYLNWYQQKPGKAPKVLIYFTSSLHSGVPSRFSGSGSGTDFTLTISSLQPEDFATYYCQQYSTVPWTFGCGTKVEIK

SEQ ID NO: 7 - protein, 495 aa, Homo sapiens
EVQLVESGGGLVQPGRSLRLSCAASGFTFDDYAMHWVRQAPGKGLEWVSGISWNSGSIGYADSVKGRFTISRDNAKNSLYLQMNSLRAEDTALYYCAKDIGGIVGAATLGDAFDIWGQGTMVTVSSASTKGPSVFPLAPSSKSTSGGTAALGCLVKDYFPEPVTVSWNSGALTSGVHTFPAVLQSSGLYSLSSVVTVPSSSLGTQTYICNVNHKPSNTKVDKKVEPKSCDKTHTGGGGGSGGGGSGGGGSEVQLVESGGGLVQPGGSLRLSCAASGYDFTHYGMNWVRQAPGKCLEWVGWINTYTGEPTYAADFKRRFTFSLDTSKSTAYLQMNSLRAEDTAVYYCAKYPYYYGTSHWYFDVWGQGTLVTVSSGGGGSGGGGSGGGGSDIQLTQSPSSLSASVGDRVTITCSASQDISNYLNWYQQKPGKAPKVLIYFTSSLHSGVPSRFSGSGSGTDFTLTISSLQPEDFATYYCQQYSTVPWTFGCGTKVEIK

SEQ ID NO: 8 - protein, 496 aa, Homo sapiens
EVQLVESGGGLVQPGRSLRLSCAASGFTFDDYAMHWVRQAPGKGLEWVSGISWNSGSIGYADSVKGRFTISRDNAKNSLYLQMNSLRAEDTALYYCAKDIGGIVGAATLGDAFDIWGQGTMVTVSSASTKGPSVFPLAPSSKSTSGGTAALGCLVKDYFPEPVTVSWNSGALTSGVHTFPAVLQSSGLYSLSSVVTVPSSSLGTQTYICNVNHKPSNTKVDKKVEPKSCGGGGGSGGGGSGGGGSEVQLVESGGGLVQPGGSLRLSCAASGYDFTHYGMNWVRQAPGKGLEWVGWINTYTGEPTYAADFKRRFTFSLDTSKSTAYLQMNSLRAEDTAVYYCAKYPYYYGTSHWYFDVWGQGTLVTVSSGGGGSGGGGSGGGGSDIQLTQSPSSLSASVGDRVTITCSASQDISNYLNWYQQKPGKAPKVLIYFTSSLHSGVPSRFSGSGSGTDFTLTISSLQPEDFATYYCQQYSTVPWTFGQGTKVEIKHHHHHH